European Patent Specification EP 3 681 901 B1, published March 27, 2024. Title: METHOD OF ENHANCING RNA EXPRESSION IN A CELL. Applicant: BioNTech RNA Pharmaceuticals GmbH et al. The sequence listing filed with the application follows.

SEQUENCE LISTING (1 sequence)

SEQ ID NO: 1 - protein, 316 aa, Toscana virus
MQSRAVILKHRSGSGHKRSLPRFYIDCDLDTFDFEKGCSLIENEFPIYINNYEVVYKSKPTLSHFLIEKEFPAVLGPGMISAVRTRLYEPTMRELYQESIHQLKRNNKKYLLSALRWPTGIPTLEFIDYYFEELLFLSEFDPGSIQRYLKLLVKASGLYNSTIEEQLVEIHRRVLIEGKKHGLTAFDLPGNDILGDICVVQAARVTRLVAKTFSKMTRDTHLMIYFSISPVELVLNKLDKKEDKRAKAKGLMSMCAARSYDYFMRTDLGFRETALSTFWAKDWPTLQETILSDKRCLKEDMRVTKWLPSPPHYPPL